European Patent Specification EP 3 389 707 B1, published August 20, 2025. Title: IMMUNOGENIC CONSTRUCT AND APPLICATIONS THEREOF. Applicant: INSTITUT NATIONAL DE LA SANTE ET DE LA RECHERCHE MEDICALE (INSERM) CENTRE NATIONAL DE LA RECHERCHE SCIENTIFIQUE (CNRS) UNIVERSITE PARIS DIDEROT PARIS 7 INSTITUT NATIONAL TRANSFUSION SANGUINE. The sequence listing filed with the application follows.

SEQUENCE LISTING (86 sequences)

SEQ ID NO: 1 - protein, 1 aa, artificial
  polyproline linker (can be repeated between 2 and 8, inclusive)
P

SEQ ID NO: 2 - protein, 1 aa, artificial
  polyglycine linker (can be repeated between 6 and 8, inclusive)
G

SEQ ID NO: 3 - protein, 5 aa, artificial
  glycine-serine linker (can be repeated between 2 and 5, inclusive)
GGGGS

SEQ ID NO: 4 - protein, 7 aa, artificial
  Alpha-helix-forming linker A(EAAAK)nA (amino acid sequence from position 2 to position 6 can be repeated between 2 and 5, inclusive)
AEAAAKA

SEQ ID NO: 5 - protein, 5 aa, artificial
  proline-alanine linker
PAPAP

SEQ ID NO: 6 - protein, 5 aa, artificial
  glycine-serine linker (repeated between 2 and 5, inclusive)
GGGGS

SEQ ID NO: 7 - protein, 20 aa, artificial
  glycine-serine linker
GGGGSGGGGSGGGGSGGGGS

SEQ ID NO: 8 - protein, 126 aa, artificial
  DARC VHH
MAQVQLQESGGGSVQAGGSLRLSCAASGYAFSSYCMAWFRQVPGKEREGVASINSDGERRGYADSVKGRFTVSRDNAKNTVYLQMNSLKPEDTAIYYCAAKRVVGGRYCGGGVSSWGQGTQVTVSS

SEQ ID NO: 9 - protein, 128 aa, artificial
  DARC VHH with restriction site
MAQVQLQESGGGSVQAGGSLRLSCAASGYAFSSYCMAWFRQVPGKEREGVASINSDGERRGYADSVKGRFTVSRDNAKNTVYLQMNSLKPEDTAIYYCAAKRVVGGRYCGGGVSSWGQGTQVTVSSAS

SEQ ID NO: 10 - protein, 123 aa, artificial
  VAR2CSA VHH
MAQVQLQESGGGLVQAGGSLRLSCAFSGSIFKMGWFRQAPGKEREFVAAIRWSGGSTYYADSVKGRFTISRDNAKNTVYLQMDSLKPEDTAVYYCAATWDLAGWNTVDEYDYWGQGTQVTVSS

SEQ ID NO: 11 - protein, 125 aa, artificial
  VAR2CSA VHH with restriction site
MAQVQLQESGGGLVQAGGSLRLSCAFSGSIFKMGWFRQAPGKEREFVAAIRWSGGSTYYADSVKGRFTISRDNAKNTVYLQMDSLKPEDTAVYYCAATWDLAGWNTVDEYDYWGQGTQVTVSSAS

SEQ ID NO: 12 - protein, 118 aa, artificial [sequence omitted]

SEQ ID NO: 13 - protein, 120 aa, artificial
  VSG VHH with restriction site
DVQLVESGGGSVQAGGSLRLSCAVSGSTYSPCTTGWYRQAPGKEREWVSSISSPGTIYYQDSVKGRFTISRDNAKNTVYLQMNSLQREDTGMYYCQIQCGVRSIREYWGQGTQVTVSSAS

SEQ ID NO: 14 - protein, 198 aa, artificial
  EPCR amino-acid 18-210
SDGLQRLHMLQISYFRDPYHVWYQGNASLGGHLTHVLEGPDTNTTIIQLQPLQEPESWARTQSGLQSYLLQFHGLVRLVHQERTLAFPLTIRCFLGCELPPEGSRAHVFFEVAVNGSSFVSFRPERALWQADTQVTSGVVTFTLQQLNAYNRTRYELREFLEDTCVQYVQKHISAENTKGSQTSRSYTSLVLGVLVGS

SEQ ID NO: 15 - protein, 176 aa, Epstein Barr virus
  MISC_FEATURE: consensus full length EBV P18 antigen
  VARIANT (2)..(2): Ala can be replaced by Ser
  VARIANT (126)..(126): Ala can be replaced by Val
  VARIANT (136)..(136): Ser can be replaced by Asn
  VARIANT (148)..(148): Ala can be absent
  VARIANT (149)..(149): Ser can be absent
  VARIANT (165)..(165): Gln can be replaced by His
MARRLPKPTLQGRLEADFPDSPLLPKFQELNQNNLPNDVFREAQRSYLVFLTSQFCYEEYVQRTFGVPRRQRAIDKRQRASVAGAGAHAHLGGSSATPVQQAQAAASAGTGALASSAPSTAVAQSATPSVSSSISSLRAATSGATAAASAAAAVDTGSGGGGQPQDTAPRGARKKQ

SEQ ID NO: 16 - protein, 162 aa, Epstein Barr virus
  MISC_FEATURE: consensus full length EBV 23 antigen
  VARIANT (39)..(39): Gln can be replaced by Arg
  VARIANT (55)..(55): Ala can be replaced by Val
  VARIANT (56)..(56): Pro can be replaced by Thr
  VARIANT (89)..(89): Asp can be replaced by Glu
  VARIANT (104)..(104): Met can be replaced by Leu
  VARIANT (106)..(106): Asn can be replaced by Lys
  VARIANT (132)..(132): Thr can be replaced by Pro
  VARIANT (134)..(134): Pro can be replaced by Leu or Ser
  VARIANT (135)..(135): Arg can be replaced by Asn or can be absent
  VARIANT (136)..(136): Glu can be replaced by Asp or can be absent
  VARIANT (137)..(137): Ser can be replaced by Pro or can be absent
  VARIANT (138)..(138): Asn can be replaced by Ser
  VARIANT (142)..(142): Ala can be replaced by Thr, Ser or Asn
  VARIANT (148)..(148): Ser can be absent
  VARIANT (149)..(149): Arg can be absent
  VARIANT (153)..(153): Arg can be replaced by Cys
  VARIANT (155)..(155): Ala can be replaced by Ser
MSAPRKVRLPSVKAVDMSMEDMAARLARLESENKALKQQVLRGGACASSTSVPSAPVPPPEPLTARQREVMITQATGRLASQAMKKIEDKVRKSVDGVTTRNEMENILQNLTLRIQVSMLGAKGQPSPGEGTRPRESNDPNATRRARSRSRGREAKKVQISD

SEQ ID NO: 17 - protein, 176 aa, Epstein Barr virus B95-8 strain
  MISC_FEATURE: wt full length EBV P18 antigen
MARRLPKPTLQGRLEADFPDSPLLPKFQELNQNNLPNDVFREAQRSYLVFLTSQFCYEEYVQRTFGVPRRQRAIDKRQRASVAGAGAHAHLGGSSATPVQQAQAAASAGTGALASSAPSTAVAQSATPSVSSSISSLRAATSGATAAASAAAAVDTGSGGGGQPHDTAPRGARKKQ

SEQ ID NO: 18 - protein, 176 aa, Epstein Barr virus alternative strain; identical to SEQ ID NO: 17
  MISC_FEATURE: wt full length EBV P18 antigen

SEQ ID NO: 19 - protein, 174 aa, Epstein Barr virus alternative strain
  MISC_FEATURE: wt full length EBV P18 antigen
MARRLPKPTLQGRLEADFPDSPLLPKFQELNQNNLPNDVFREAQRSYLVFLTSQFCYEEYVQRTFGVPRRQRAIDKRQRASVAGAGAHAHLGGSSATPVQQAQAAASAGTGALASSAPSTAVAQSATPSVSSSISSLRAATSGATAAAAAAVDTGSGGGGQPQDTAPRGARKKQ

SEQ ID NO: 20 - protein, 176 aa, Epstein Barr virus alternative strain
  MISC_FEATURE: wt full length EBV P18 antigen
MARRLPKPTLQGRLEADFPDSPLLPKFQELNQNNLPNDVFREAQRSYLVFLTSQFCYEEYVQRTFGVPRRQRAIDKRQRASVAGAGAHAHLGGSSATPVQQAQAAASAGTGALASSAPSTAVAQSATPSVSSSISNLRAATSGATAAASAAAAVDTGSGGGGQPQDTAPRGARKKQ

SEQ ID NO: 21 - protein, 176 aa, Epstein Barr virus alternative strain
  MISC_FEATURE: wt full length EBV P18 antigen
MARRLPKPTLQGRLEADFPDSPLLPKFQELNQNNLPNDVFREAQRSYLVFLTSQFCYEEYVQRTFGVPRRQRAIDKRQRASVAGAGAHAHLGGSSATPVQQAQAAASAGTGALASSAPSTAVAQSVTPSVSSSISSLRAATSGATAAASAAAAVDTGSGGGGQPQDTAPRGARKKQ

SEQ ID NO: 22 - protein, 176 aa, Epstein Barr virus alternative strain
  MISC_FEATURE: wt full length EBV P18 antigen
MSRRLPKPTLQGRLEADFPDSPLLPKFQELNQNNLPNDVFREAQRSYLVFLTSQFCYEEYVQRTFGVPRRQRAIDKRQRASVAGAGAHAHLGGSSATPVQQAQAAASAGTGALASSAPSTAVAQSATPSVSSSISSLRAATSGATAAASAAAAVDTGSGGGGQPQDTAPRGARKKQ

SEQ ID NO: 23 - protein, 162 aa, Epstein Barr virus B95-8 strain; identical to SEQ ID NO: 16
  MISC_FEATURE: wt full length EBV P23 antigen

SEQ ID NO: 24 - protein, 162 aa, Epstein Barr virus alternative strain
  MISC_FEATURE: wt full length EBV P23 antigen
MSAPRKVRLPSVKAVDMSMEDMAARLARLESENKALKQQVLRGGACASSTSVPSAPVPPPEPLTARQREVMITQATGRLASQAMKKIEDKVRKSVDGVTTRNEMENILQNLTLRIQVSMLGAKGQPSPGEGTRLRESNDPNATRRARSRSRGREAKKVQISD

SEQ ID NO: 25 - protein, 159 aa, Epstein Barr virus alternative strain
  MISC_FEATURE: wt full length EBV P23 antigen
MSAPRKVRLPSVKAVDMSMEDMAARLARLESENKALKQQVLRGGACASSTSVPSAPVPPPEPLTARQREVMITQATGRLASQAMKKIEDKVRKSVDGVTTRNEMENILQNLTLRIQVSMLGAKGQPSPGEGTRPNDPNATRRARSRSRGREAKKVQISD

SEQ ID NO: 26 - protein, 159 aa, Epstein Barr virus alternative strain
  MISC_FEATURE: wt full length EBV P23 antigen
MSAPRKVRLPSVKAVDMSMEDMAARLARLESENKALKQQVLRGGACASSTSVPSAPVPPPEPLTARQREVMITQATGRLASQAMKKIEDKVRKSVDGVTTRNEMEKILQNLTLRIQVSMLGAKGQPSPGEGTRPNDPNATRRARSRSRGREAKKVQISD

SEQ ID NO: 27 - protein, 162 aa, Epstein Barr virus alternative strain
  MISC_FEATURE: wt full length EBV P23 antigen
MSAPRKVRLPSVKAVDMSMEDMAARLARLESENKALKQQVLRGGACASSTSVPSAPVPPPEPLTARQREVMITQATGRLASQAMKKIEDKVRKSVDGVTTRNELENILQNLTLRIQVSMLGAKGQPSPGEGTRPRESSDPNATRRARSRSRGREAKKVQISD

SEQ ID NO: 28 - protein, 162 aa, Epstein Barr virus alternative strain
  MISC_FEATURE: wt full length EBV P23 antigen
MSAPRKVRLPSVKAVDMSMEDMAARLARLESENKALKQQVLRGGACASSTSVPSVPVPPPEPLTARQREVMITQATGRLASQAMKKIEDKVRKSVDGVTTRNEMENILQNLTLRIQVSMLGAKGQPSPGEGTRPRESNDPNATRRARSRSRGREAKKVQISD

SEQ ID NO: 29 - protein, 159 aa, Epstein Barr virus alternative strain
  MISC_FEATURE: wt full length EBV P23 antigen
MSAPRKVRLPSVKAVDMSMEDMAARLARLESENKALKQRVLRGGACASSTSVPSAPVPPPEPLTARQREVMITQATGRLASQAMKKIEDKVRKSVDGVTTRNEMENILQNLTLRIQVSMLGAKGQPSPGEGTRPNDPNATRRARSRSRGREAKKVQISD

SEQ ID NO: 30 - protein, 159 aa, Epstein Barr virus alternative strain
  MISC_FEATURE: wt full length EBV P23 antigen
MSAPRKVRLPSVKAVDMSMEDMAARLARLESENKALKQQVLRGGACASSTSVPSATVPPPEPLTARQREVMITQATGRLASQAMKKIEDKVRKSVDGVTTRNEMENILQNLTLRIQVSMLGAKGQPSPGEGTRPNDPNATRRARSRSRGREAKKVQISD

SEQ ID NO: 31 - protein, 160 aa, Epstein Barr virus alternative strain
  MISC_FEATURE: wt full length EBV P23 antigen
MSAPRKVRLPSVKAVDMSMEDMAARLARLESENKALKQQVLRGGACASSTSVPSAPVPPPEPLTARQREVMITQATGRLASQAMKKIEDKVRKSVDGVTTRNEMENILQNLTLRIQVSMLGAKGQPSPGEGTRPRESNDPNATRRARSRGREAKKVQISD

SEQ ID NO: 32 - protein, 162 aa, Epstein Barr virus alternative strain
  MISC_FEATURE: wt full length EBV P23 antigen
MSAPRKVRLPSVKAVDMSMEDMAARLARLESENKALKQQVLRGGACASSTSVPSAPVPPPEPLTARQREVMITQATGRLASQAMKKIEDKVRKSVDGVTTRNEMENILQNLTLRIQVSMLGAKGQPSPGEGTRSRESNDPNATRRARSRSRGREAKKVQISD

SEQ ID NO: 33 - protein, 162 aa, Epstein Barr virus alternative strain
  MISC_FEATURE: wt full length EBV P23 antigen
MSAPRKVRLPSVKAVDMSMEDMAARLARLESENKALKQQVLRGGACASSTSVPSAPVPPPEPLTARQREVMITQATGRLASQAMKKIEDKVRKSVDGVTTRNEMENILQNLTLRIQVSMLGAKGQPSPGEGPRPRESNDPNATRRARSRSRGREAKKVQISD

SEQ ID NO: 34 - protein, 162 aa, Epstein Barr virus alternative strain
  MISC_FEATURE: wt full length EBV P23 antigen
MSAPRKVRLPSVKAVDMSMEDMAARLARLESENKALKQQVLRGGACASSTSVPSAPVPPPEPLTARQREVMITQATGRLASQAMKKIEDKVRKSVDGVTTRNEMENILQNLTLRIQVSMLGAKGQPSPGEGTRPRESNDPNTTRRARSRSRGREAKKVQISD

SEQ ID NO: 35 - protein, 159 aa, Epstein Barr virus alternative strain; identical to SEQ ID NO: 26
  MISC_FEATURE: wt full length EBV P23 antigen

SEQ ID NO: 36 - protein, 162 aa, Epstein Barr virus alternative strain
  MISC_FEATURE: wt full length EBV P23 antigen
MSAPRKVRLPSVKAVDMSMEDMAARLARLESENKALKQQVLRGGACASSTSVPSAPVPPPEPLTARQREVMITQATGRLASQAMKKIEEKVRKSVDGVTTRNEMENILQNLTLRIQVSMLGAKGQPSPGEGTRPRESNDPNATRRARSRSRGREAKKVQISD

SEQ ID NO: 37 - protein, 162 aa, Epstein Barr virus alternative strain
  MISC_FEATURE: wt full length EBV P23 antigen
MSAPRKVRLPSVKAVDMSMEDMAARLARLESENKALKQQVLRGGACASSTSVPSAPVPPPEPLTARQREVMITQATGRLASQAMKKIEDKVRKSVDGVTTRNEMENILQNLTLRIQVSMLGAKGQPSPGEGTRPRESNDPNSTRRARSRSRGREAKKVQISD

SEQ ID NO: 38 - protein, 162 aa, Epstein Barr virus alternative strain
  MISC_FEATURE: wt full length EBV P23 antigen
MSAPRKVRLPSVKAVDMSMEDMAARLARLESENKALKQQVLRGGACASSTSVPSAPVPPPEPLTARQREVMITQATGRLASQAMKKIEDKVRKSVDGVTTRNEMENILQNLTLRIQVSMLGAKGQPSPGEGTRLRESNDPNATRRARSRSRGCESKKVQISD

SEQ ID NO: 39 - protein, 176 aa, artificial
  consensus EBV mutated P18 antigen (C56S)*
  VARIANT (2)..(2): Ala can be replaced by Ser
  VARIANT (126)..(126): Ala can be replaced by Val
  VARIANT (136)..(136): Ser can be replaced by Asn
  VARIANT (148)..(148): Ala can be absent
  VARIANT (149)..(149): Ser can be absent
  VARIANT (165)..(165): Gln can be replaced by His
MARRLPKPTLQGRLEADFPDSPLLPKFQELNQNNLPNDVFREAQRSYLVFLTSQFSYEEYVQRTFGVPRRQRAIDKRQRASVAGAGAHAHLGGSSATPVQQAQAAASAGTGALASSAPSTAVAQSATPSVSSSISSLRAATSGATAAASAAAAVDTGSGGGGQPQDTAPRGARKKQ

SEQ ID NO: 40 - protein, 162 aa, artificial
  consensus EBV mutated P23 antigen (C46S)*
  VARIANT (39)..(39): Gln can be replaced by Arg
  VARIANT (55)..(55): Ala can be replaced by Val
  VARIANT (56)..(56): Pro can be replaced by Thr
  VARIANT (89)..(89): Asp can be replaced by Glu
  VARIANT (104)..(104): Met can be replaced by Leu
  VARIANT (106)..(106): Asn can be replaced by Lys
  VARIANT (132)..(132): Thr can be replaced by Pro
  VARIANT (134)..(134): Pro can be replaced by Leu or Ser
  VARIANT (135)..(135): Arg can be replaced by Asn or can be absent
  VARIANT (136)..(136): Glu can be replaced by Asp or can be absent
  VARIANT (137)..(137): Ser can be replaced by Pro or can be absent
  VARIANT (138)..(138): Asn can be replaced by Ser
  VARIANT (142)..(142): Ala can be replaced by Thr, Ser or Asn
  VARIANT (148)..(148): Ser can be absent
  VARIANT (149)..(149): Arg can be absent
  VARIANT (153)..(153): Arg can be replaced by Cys
  VARIANT (155)..(155): Ala can be replaced by Ser
MSAPRKVRLPSVKAVDMSMEDMAARLARLESENKALKQQVLRGGASASSTSVPSAPVPPPEPLTARQREVMITQATGRLASQAMKKIEDKVRKSVDGVTTRNEMENILQNLTLRIQVSMLGAKGQPSPGEGTRPRESNDPNATRRARSRSRGREAKKVQISD

SEQ ID NO: 41 - protein, 176 aa, artificial
  EBV mutated P18 antigen (C56S)*
MARRLPKPTLQGRLEADFPDSPLLPKFQELNQNNLPNDVFREAQRSYLVFLTSQFSYEEYVQRTFGVPRRQRAIDKRQRASVAGAGAHAHLGGSSATPVQQAQAAASAGTGALASSAPSTAVAQSATPSVSSSISSLRAATSGATAAASAAAAVDTGSGGGGQPHDTAPRGARKKQ

SEQ ID NO: 42 - protein, 162 aa, artificial; identical to SEQ ID NO: 40
  EBV mutated P23 antigen (C46S)*

SEQ ID NO: 43 - protein, 23 aa, artificial
  consensus EBV P18 antigen fragment F4
  VARIANT (12)..(12): Gln can be replaced by His
VDTGSGGGGQPQDTAPRGARKKQ

SEQ ID NO: 44 - protein, 94 aa, artificial
  consensus EBV P18 antigen fragment F3'
  VARIANT (44)..(44): Ala can be replaced by Val
  VARIANT (54)..(54): Ser can be replaced by Asn
  VARIANT (66)..(66): Ala can be absent
  VARIANT (67)..(67): Ser can be absent
  VARIANT (83)..(83): Gln can be replaced by His
AGAGAHAHLGGSSATPVQQAQAAASAGTGALASSAPSTAVAQSATPSVSSSISSLRAATSGATAAASAAAAVDTGSGGGGQPQDTAPRGARKKQ

SEQ ID NO: 45 - protein, 84 aa, artificial
  consensus EBV P18 antigen fragment F2-F4
  VARIANT (57)..(57): Ala can be replaced by Val
  VARIANT (67)..(67): Ser can be replaced by Asn
  VARIANT (79)..(79): Ala can be absent
  VARIANT (80)..(80): Ser can be absent
RQRAIDKRQRASVAGAGAHAHLGGSSATPVQQAQAAASAGTGALASSAPSTAVAQSATPSVSSSISSLRAATSGATAAASAAAA

SEQ ID NO: 46 - protein, 71 aa, artificial
  Consensus EBV P18 antigen fragment F3'-F4
  VARIANT (44)..(44): Ala can be replaced by Val
  VARIANT (54)..(54): Ser can be replaced by Asn
  VARIANT (66)..(66): Ala can be absent
  VARIANT (67)..(67): Ser can be absent
AGAGAHAHLGGSSATPVQQAQAAASAGTGALASSAPSTAVAQSATPSVSSSISSLRAATSGATAAASAAAA

SEQ ID NO: 47 - protein, 20 aa, artificial
  Consensus EBV P18 antigen fragment P18F5
  VARIANT (2)..(2): Ala can be replaced by Val
  VARIANT (12)..(12): Ser can be replaced by Asn
SATPSVSSSISSLRAATSGA

SEQ ID NO: 48 - protein, 10 aa, artificial
  Consensus EBV P18 antigen fragment P18F6
  VARIANT (8)..(8): Ser can be replaced by Asn
SVSSSISSLR

SEQ ID NO: 49 - protein, 107 aa, artificial
  consensus EBV P18 antigen fragment F2
  VARIANT (57)..(57): Ala can be replaced by Val
  VARIANT (67)..(67): Ser can be replaced by Asn
  VARIANT (79)..(79): Ala can be absent
  VARIANT (80)..(80): Ser can be absent
  VARIANT (96)..(96): Gln can be replaced by His
RQRAIDKRQRASVAGAGAHAHLGGSSATPVQQAQAAASAGTGALASSAPSTAVAQSATPSVSSSISSLRAATSGATAAASAAAAVDTGSGGGGQPQDTAPRGARKKQ

SEQ ID NO: 50 - protein, 60 aa, artificial
  consensus EBV P23 antigen fragment F3
  VARIANT (2)..(2): Met can be replaced by Leu
  VARIANT (4)..(4): Asn can be replaced by Lys
  VARIANT (30)..(30): Thr can be replaced by Pro
  VARIANT (32)..(32): Pro can be replaced by Leu or Ser
  VARIANT (33)..(33): Arg can be replaced by Asn or can be absent
  VARIANT (34)..(34): Glu can be replaced by Asp or can be absent
  VARIANT (35)..(35): Ser can be replaced by Pro or can be absent
  VARIANT (36)..(36): Asn can be replaced by Ser
  VARIANT (40)..(40): Ala can be replaced by Thr, Ser or Asn
  VARIANT (46)..(46): Ser can be absent
  VARIANT (47)..(47): Arg can be absent
  VARIANT (51)..(51): Arg can be replaced by Cys
  VARIANT (53)..(53): Ala can be replaced by Ser
EMENILQNLTLRIQVSMLGAKGQPSPGEGTRPRESNDPNATRRARSRSRGREAKKVQISD

SEQ ID NO: 51 - protein, 88 aa, artificial
  consensus EBV P23 antigen fragment F2
  VARIANT (15)..(15): Asp can be replaced by Glu
  VARIANT (30)..(30): Met can be replaced by Leu
  VARIANT (32)..(32): Asn can be replaced by Lys
  VARIANT (58)..(58): Thr can be replaced by Pro
  VARIANT (60)..(60): Pro can be replaced by Leu or Ser
  VARIANT (61)..(61): Arg can be replaced by Asn or can be absent
  VARIANT (62)..(62): Glu can be replaced by Asp or can be absent
  VARIANT (63)..(63): Ser can be replaced by Pro or can be absent
  VARIANT (64)..(64): Asn can be replaced by Ser
  VARIANT (68)..(68): Ala can be replaced by Thr, Ser or Asn
  VARIANT (74)..(74): Ser can be absent
  VARIANT (75)..(75): Arg can be absent
  VARIANT (79)..(79): Arg can be replaced by Cys
  VARIANT (81)..(81): Ala can be replaced by Ser
ATGRLASQAMKKIEDKVRKSVDGVTTRNEMENILQNLTLRIQVSMLGAKGQPSPGEGTRPRESNDPNATRRARSRSRGREAKKVQISD

SEQ ID NO: 52 - protein, 23 aa, artificial
  EBV P18 antigen fragment F4
VDTGSGGGGQPHDTAPRGARKKQ

SEQ ID NO: 53 - protein, 92 aa, artificial
  EBV P18 antigen fragment F3'
AGAHAHLGGSSATPVQQAQAAASAGTGALASSAPSTAVAQSATPSVSSSISSLRAATSGATAAASAAAAVDTGSGGGGQPHDTAPRGARKKQ

SEQ ID NO: 54 - protein, 84 aa, artificial; identical to SEQ ID NO: 45
  EBV P18 antigen fragment F2-F4

SEQ ID NO: 55 - protein, 71 aa, artificial; identical to SEQ ID NO: 46
  EBV P18 antigen fragment F3'-F4

SEQ ID NO: 56 - protein, 20 aa, artificial
  EBV P18 antigen fragment P18F5
SATPSVSSSISSLRAATSGA

SEQ ID NO: 57 - protein, 10 aa, artificial
  EBV P18 antigen fragment P18F6
SVSSSISSLR

SEQ ID NO: 58 - protein, 107 aa, artificial
  EBV P18 antigen fragment F2
RQRAIDKRQRASVAGAGAHAHLGGSSATPVQQAQAAASAGTGALASSAPSTAVAQSATPSVSSSISSLRAATSGATAAASAAAAVDTGSGGGGQPHDTAPRGARKKQ

SEQ ID NO: 59 - protein, 60 aa, artificial; identical to SEQ ID NO: 50
  EBV P23 antigen fragment F3

SEQ ID NO: 60 - protein, 88 aa, artificial; identical to SEQ ID NO: 51
  EBV P23 antigen fragment F2

SEQ ID NO: 61 - protein, 324 aa, artificial
  conjugate DARC VHH (with restriction site)  - glycine serine linker - EBV wt full length P18 antigen
MAQVQLQESGGGSVQAGGSLRLSCAASGYAFSSYCMAWFRQVPGKEREGVASINSDGERRGYADSVKGRFTVSRDNAKNTVYLQMNSLKPEDTAIYYCAAKRVVGGRYCGGGVSSWGQGTQVTVSSASGGGGSGGGGSGGGGSGGGGSMARRLPKPTLQGRLEADFPDSPLLPKFQELNQNNLPNDVFREAQRSYLVFLTSQFCYEEYVQRTFGVPRRQRAIDKRQRASVAGAGAHAHLGGSSATPVQQAQAAASAGTGALASSAPSTAVAQSATPSVSSSISSLRAATSGATAAASAAAAVDTGSGGGGQPHDTAPRGARKKQ

SEQ ID NO: 62 - protein, 324 aa, artificial
  conjugate DARC VHH (with restriction site) - glycine serine linker - EBV mutated P18 antigen (C56S)*
MAQVQLQESGGGSVQAGGSLRLSCAASGYAFSSYCMAWFRQVPGKEREGVASINSDGERRGYADSVKGRFTVSRDNAKNTVYLQMNSLKPEDTAIYYCAAKRVVGGRYCGGGVSSWGQGTQVTVSSASGGGGSGGGGSGGGGSGGGGSMARRLPKPTLQGRLEADFPDSPLLPKFQELNQNNLPNDVFREAQRSYLVFLTSQFSYEEYVQRTFGVPRRQRAIDKRQRASVAGAGAHAHLGGSSATPVQQAQAAASAGTGALASSAPSTAVAQSATPSVSSSISSLRAATSGATAAASAAAAVDTGSGGGGQPHDTAPRGARKKQ

SEQ ID NO: 63 - protein, 304 aa, artificial
  conjugate DARC VHH (with restriction site) - EBV mutated P18 antigen (C56S)*
MAQVQLQESGGGSVQAGGSLRLSCAASGYAFSSYCMAWFRQVPGKEREGVASINSDGERRGYADSVKGRFTVSRDNAKNTVYLQMNSLKPEDTAIYYCAAKRVVGGRYCGGGVSSWGQGTQVTVSSASMARRLPKPTLQGRLEADFPDSPLLPKFQELNQNNLPNDVFREAQRSYLVFLTSQFSYEEYVQRTFGVPRRQRAIDKRQRASVAGAGAHAHLGGSSATPVQQAQAAASAGTGALASSAPSTAVAQSATPSVSSSISSLRAATSGATAAASAAAAVDTGSGGGGQPHDTAPRGARKKQ

SEQ ID NO: 64 - protein, 235 aa, artificial
  conjugate DARC VHH (with restriction site) - EBV P18 antigen fragment F2
MAQVQLQESGGGSVQAGGSLRLSCAASGYAFSSYCMAWFRQVPGKEREGVASINSDGERRGYADSVKGRFTVSRDNAKNTVYLQMNSLKPEDTAIYYCAAKRVVGGRYCGGGVSSWGQGTQVTVSSASRQRAIDKRQRASVAGAGAHAHLGGSSATPVQQAQAAASAGTGALASSAPSTAVAQSATPSVSSSISSLRAATSGATAAASAAAAVDTGSGGGGQPHDTAPRGARKKQ

SEQ ID NO: 65 - protein, 220 aa, artificial
  conjugate DARC VHH (with restriction site) - EBV P18 antigen fragment F3'
MAQVQLQESGGGSVQAGGSLRLSCAASGYAFSSYCMAWFRQVPGKEREGVASINSDGERRGYADSVKGRFTVSRDNAKNTVYLQMNSLKPEDTAIYYCAAKRVVGGRYCGGGVSSWGQGTQVTVSSASAGAHAHLGGSSATPVQQAQAAASAGTGALASSAPSTAVAQSATPSVSSSISSLRAATSGATAAASAAAAVDTGSGGGGQPHDTAPRGARKKQ

SEQ ID NO: 66 - protein, 151 aa, artificial
  conjugate DARC VHH (with restriction site) - EBV P18 antigen fragment F4
MAQVQLQESGGGSVQAGGSLRLSCAASGYAFSSYCMAWFRQVPGKEREGVASINSDGERRGYADSVKGRFTVSRDNAKNTVYLQMNSLKPEDTAIYYCAAKRVVGGRYCGGGVSSWGQGTQVTVSSASVDTGSGGGGQPHDTAPRGARKKQ

SEQ ID NO: 67 - protein, 232 aa, artificial
  conjugate VAR2CSA VHH (with restriction site)- EBV P18 antigen fragment F2
MAQVQLQESGGGLVQAGGSLRLSCAFSGSIFKMGWFRQAPGKEREFVAAIRWSGGSTYYADSVKGRFTISRDNAKNTVYLQMDSLKPEDTAVYYCAATWDLAGWNTVDEYDYWGQGTQVTVSSASRQRAIDKRQRASVAGAGAHAHLGGSSATPVQQAQAAASAGTGALASSAPSTAVAQSATPSVSSSISSLRAATSGATAAASAAAAVDTGSGGGGQPHDTAPRGARKKQ

SEQ ID NO: 68 - protein, 217 aa, artificial
  conjugate VAR2CSA VHH (with restriction site)- EBV P18 antigen fragment F3'
MAQVQLQESGGGLVQAGGSLRLSCAFSGSIFKMGWFRQAPGKEREFVAAIRWSGGSTYYADSVKGRFTISRDNAKNTVYLQMDSLKPEDTAVYYCAATWDLAGWNTVDEYDYWGQGTQVTVSSASAGAHAHLGGSSATPVQQAQAAASAGTGALASSAPSTAVAQSATPSVSSSISSLRAATSGATAAASAAAAVDTGSGGGGQPHDTAPRGARKKQ

SEQ ID NO: 69 - protein, 148 aa, artificial
  conjugate VAR2CSA VHH (with restriction site) - EBV P18 antigen fragment F4
MAQVQLQESGGGLVQAGGSLRLSCAFSGSIFKMGWFRQAPGKEREFVAAIRWSGGSTYYADSVKGRFTISRDNAKNTVYLQMDSLKPEDTAVYYCAATWDLAGWNTVDEYDYWGQGTQVTVSSASVDTGSGGGGQPHDTAPRGARKKQ

SEQ ID NO: 70 - protein, 310 aa, artificial
  conjugate DARC VHH (with restriction site) - glycine serine linker - EBV wt full length P23 antigen
MAQVQLQESGGGSVQAGGSLRLSCAASGYAFSSYCMAWFRQVPGKEREGVASINSDGERRGYADSVKGRFTVSRDNAKNTVYLQMNSLKPEDTAIYYCAAKRVVGGRYCGGGVSSWGQGTQVTVSSASGGGGSGGGGSGGGGSGGGGSMSAPRKVRLPSVKAVDMSMEDMAARLARLESENKALKQQVLRGGACASSTSVPSAPVPPPEPLTARQREVMITQATGRLASQAMKKIEDKVRKSVDGVTTRNEMENILQNLTLRIQVSMLGAKGQPSPGEGTRPRESNDPNATRRARSRSRGREAKKVQISD

SEQ ID NO: 71 - protein, 310 aa, artificial
  conjugate DARC VHH (with restriction site) - glycine serine linker - EBV mutated P23 antigen (C46S)*
MAQVQLQESGGGSVQAGGSLRLSCAASGYAFSSYCMAWFRQVPGKEREGVASINSDGERRGYADSVKGRFTVSRDNAKNTVYLQMNSLKPEDTAIYYCAAKRVVGGRYCGGGVSSWGQGTQVTVSSASGGGGSGGGGSGGGGSGGGGSMSAPRKVRLPSVKAVDMSMEDMAARLARLESENKALKQQVLRGGASASSTSVPSAPVPPPEPLTARQREVMITQATGRLASQAMKKIEDKVRKSVDGVTTRNEMENILQNLTLRIQVSMLGAKGQPSPGEGTRPRESNDPNATRRARSRSRGREAKKVQISD

SEQ ID NO: 72 - protein, 290 aa, artificial
  conjugate DARC VHH (with restriction site) - EBV mutated P23 antigen(C46S)*
MAQVQLQESGGGSVQAGGSLRLSCAASGYAFSSYCMAWFRQVPGKEREGVASINSDGERRGYADSVKGRFTVSRDNAKNTVYLQMNSLKPEDTAIYYCAAKRVVGGRYCGGGVSSWGQGTQVTVSSASMSAPRKVRLPSVKAVDMSMEDMAARLARLESENKALKQQVLRGGASASSTSVPSAPVPPPEPLTARQREVMITQATGRLASQAMKKIEDKVRKSVDGVTTRNEMENILQNLTLRIQVSMLGAKGQPSPGEGTRPRESNDPNATRRARSRSRGREAKKVQISD

SEQ ID NO: 73 - protein, 216 aa, artificial
  conjugate DARC VHH (with restriction site) - EBV P23 antigen fragment F2
MAQVQLQESGGGSVQAGGSLRLSCAASGYAFSSYCMAWFRQVPGKEREGVASINSDGERRGYADSVKGRFTVSRDNAKNTVYLQMNSLKPEDTAIYYCAAKRVVGGRYCGGGVSSWGQGTQVTVSSASATGRLASQAMKKIEDKVRKSVDGVTTRNEMENILQNLTLRIQVSMLGAKGQPSPGEGTRPRESNDPNATRRARSRSRGREAKKVQISD

SEQ ID NO: 74 - protein, 188 aa, artificial
  conjugate DARC VHH (with restriction site) - EBV P23 antigen fragment F3
MAQVQLQESGGGSVQAGGSLRLSCAASGYAFSSYCMAWFRQVPGKEREGVASINSDGERRGYADSVKGRFTVSRDNAKNTVYLQMNSLKPEDTAIYYCAAKRVVGGRYCGGGVSSWGQGTQVTVSSASEMENILQNLTLRIQVSMLGAKGQPSPGEGTRPRESNDPNATRRARSRSRGREAKKVQISD

SEQ ID NO: 75 - protein, 72 aa, artificial
  Consensus EBV P18 antigen fragment F3
  VARIANT (22)..(22): Ala can be replaced by Val
  VARIANT (32)..(32): Ser can be replaced by Asn
  VARIANT (44)..(44): Ala can be absent
  VARIANT (45)..(45): Ser can be absent
  VARIANT (61)..(61): Gln can be replaced by His
AASAGTGALASSAPSTAVAQSATPSVSSSISSLRAATSGATAAASAAAAVDTGSGGGGQPQDTAPRGARKKQ

SEQ ID NO: 76 - protein, 72 aa, artificial
  EBV P18 antigen fragment F3
AASAGTGALASSAPSTAVAQSATPSVSSSISSLRAATSGATAAASAAAAVDTGSGGGGQPHDTAPRGARKKQ

SEQ ID NO: 77 - protein, 200 aa, artificial
  conjugate DARC VHH (with restriction site) - EBV P18 antigen fragment F3
MAQVQLQESGGGSVQAGGSLRLSCAASGYAFSSYCMAWFRQVPGKEREGVASINSDGERRGYADSVKGRFTVSRDNAKNTVYLQMNSLKPEDTAIYYCAAKRVVGGRYCGGGVSSWGQGTQVTVSSASAASAGTGALASSAPSTAVAQSATPSVSSSISSLRAATSGATAAASAAAAVDTGSGGGGQPHDTAPRGARKKQ

SEQ ID NO: 78 - protein, 197 aa, artificial
  conjugate VAR2CSA VHH (with restriction site)- EBV P18 antigen fragment F3
MAQVQLQESGGGLVQAGGSLRLSCAFSGSIFKMGWFRQAPGKEREFVAAIRWSGGSTYYADSVKGRFTISRDNAKNTVYLQMDSLKPEDTAVYYCAATWDLAGWNTVDEYDYWGQGTQVTVSSASAASAGTGALASSAPSTAVAQSATPSVSSSISSLRAATSGATAAASAAAAVDTGSGGGGQPHDTAPRGARKKQ

SEQ ID NO: 79 - protein, 270 aa, artificial
  conjugate EPCR amino-acid 18-210 - EBV P18 antigen fragment F3
SDGLQRLHMLQISYFRDPYHVWYQGNASLGGHLTHVLEGPDTNTTIIQLQPLQEPESWARTQSGLQSYLLQFHGLVRLVHQERTLAFPLTIRCFLGCELPPEGSRAHVFFEVAVNGSSFVSFRPERALWQADTQVTSGVVTFTLQQLNAYNRTRYELREFLEDTCVQYVQKHISAENTKGSQTSRSYTSLVLGVLVGSAASAGTGALASSAPSTAVAQSATPSVSSSISSLRAATSGATAAASAAAAVDTGSGGGGQPHDTAPRGARKKQ

SEQ ID NO: 80 - protein, 245 aa, artificial
  Anti-CD20 scFv
MAQAYLQQSGAELVRPGASVKMSCKASGYTFTSYNMHWVKQTPRQGLEWIGAIYPGNGDTSYNQKFKGKATLTVDKSSSTAYMQLSSLTSEDSAVYFCARVVYYSNSYWYFDVWGTGTTVTVSSGGGGSGGGGSGGGGSDIVLSQSPAILSASPGEKVTMTCRASSSVSYMHWYQQKPGSSPKPWIYAPSNLASGVPARFSGSGSGTSYSLTISRVEAEDAATYYCQQWSFNPPTFGAGTKLELK

SEQ ID NO: 81 - protein, 319 aa, artificial
  Anti-CD20 scFv - EBV P18 antigen fragment F3
MAQAYLQQSGAELVRPGASVKMSCKASGYTFTSYNMHWVKQTPRQGLEWIGAIYPGNGDTSYNQKFKGKATLTVDKSSSTAYMQLSSLTSEDSAVYFCARVVYYSNSYWYFDVWGTGTTVTVSSGGGGSGGGGSGGGGSDIVLSQSPAILSASPGEKVTMTCRASSSVSYMHWYQQKPGSSPKPWIYAPSNLASGVPARFSGSGSGTSYSLTISRVEAEDAATYYCQQWSFNPPTFGAGTKLELKASAASAGTGALASSAPSTAVAQSATPSVSSSISSLRAATSGATAAASAAAAVDTGSGGGGQPHDTAPRGARKKQ

SEQ ID NO: 82 - protein, 1016 aa, artificial
  VAR2CSA
MDKSSIANKIEAYLGAKSDDSKIDQSLKADPSEVQYYGSGGDGYYLRKNICKITVNHSDSGTNDPCDRIPPPYGDNDQWKCAIILSKVSEKPENVFVPPRRQRMCINNLEKLNVDKIRDKHAFLADVLLTARNEGERIVQNHPDTNSSNVCNALERSFADIADIIRGTDLWKGTNSNLEQNLKQMFAKIRENDKVLQDKYPKDQNYRKLREDWWNANRQKVWEVITCGARSNDLLIKRGWRTSGKSNGDNKLELCRKCGHYEEKVPTKLDYVPQFLRWLTEWIEDFYREKQNLIDDMERHREECTSEDHKSKEGTSYCSTCKDKCKKYCECVKKWKSEWENQKNKYTELYQQNKNETSQKNTSRYDDYVKDFFKKLEANYSSLENYIKGDPYFAEYATKLSFILNSSDANNPSEKIQKNNDEVCNCNESGIASVEQEQISDPSSNKTCITHSSIKANKKKVCKHVKLGVRENDKDLRVCVIEHTSLSGVENCCCQDFLRILQENCSDNKSGSSSNGSCNNKNQEACEKNLEKVLASLTNCYKCDKCKSEQSKKNNKNWIWKKSSGKEGGLQKEYANTIGLPPRTQSLCLVVCLDEKGKKTQELKNIRTNSELLKEWIIAAFHEGKNLKPSHEKKNDDNGKKLCKALEYSFADYGDLIKGTSIWDNEYTKDLELNLQKIFGKLFRKYIKKNNTAEQDTSYSSLDELRESWWNTNKKYIWLAMKHGAGMNSTTCCGDGSVTGSGSSCDDIPTIDLIPQYLRFLQEWVEHFCKQRQEKVKPVIENCKSCKESGGTCNGECKTECKNKCEVYKKFIEDCKGGDGTAGSSWVKRWDQIYKRYSKYIEDAKRNRKAGTKNCGPSSTTNAAENKCVQSDIDSFFKHLIDIGLTTPSSYLSIVLDDNICGADKAPWTTYTTYTTTEKCNKETDKSKLQQCNTAVVVNVPSPLGNTPHGYKYACQCKIPTNEETCDDRKEYMNQWSCGSARTMKRGYKNDNYELCKYNGVDVKPTTVRSNSSKLD

SEQ ID NO: 83 - protein, 1088 aa, artificial
  VAR2CSA - EBV P18 antigen fragment F3
MDKSSIANKIEAYLGAKSDDSKIDQSLKADPSEVQYYGSGGDGYYLRKNICKITVNHSDSGTNDPCDRIPPPYGDNDQWKCAIILSKVSEKPENVFVPPRRQRMCINNLEKLNVDKIRDKHAFLADVLLTARNEGERIVQNHPDTNSSNVCNALERSFADIADIIRGTDLWKGTNSNLEQNLKQMFAKIRENDKVLQDKYPKDQNYRKLREDWWNANRQKVWEVITCGARSNDLLIKRGWRTSGKSNGDNKLELCRKCGHYEEKVPTKLDYVPQFLRWLTEWIEDFYREKQNLIDDMERHREECTSEDHKSKEGTSYCSTCKDKCKKYCECVKKWKSEWENQKNKYTELYQQNKNETSQKNTSRYDDYVKDFFKKLEANYSSLENYIKGDPYFAEYATKLSFILNSSDANNPSEKIQKNNDEVCNCNESGIASVEQEQISDPSSNKTCITHSSIKANKKKVCKHVKLGVRENDKDLRVCVIEHTSLSGVENCCCQDFLRILQENCSDNKSGSSSNGSCNNKNQEACEKNLEKVLASLTNCYKCDKCKSEQSKKNNKNWIWKKSSGKEGGLQKEYANTIGLPPRTQSLCLVVCLDEKGKKTQELKNIRTNSELLKEWIIAAFHEGKNLKPSHEKKNDDNGKKLCKALEYSFADYGDLIKGTSIWDNEYTKDLELNLQKIFGKLFRKYIKKNNTAEQDTSYSSLDELRESWWNTNKKYIWLAMKHGAGMNSTTCCGDGSVTGSGSSCDDIPTIDLIPQYLRFLQEWVEHFCKQRQEKVKPVIENCKSCKESGGTCNGECKTECKNKCEVYKKFIEDCKGGDGTAGSSWVKRWDQIYKRYSKYIEDAKRNRKAGTKNCGPSSTTNAAENKCVQSDIDSFFKHLIDIGLTTPSSYLSIVLDDNICGADKAPWTTYTTYTTTEKCNKETDKSKLQQCNTAVVVNVPSPLGNTPHGYKYACQCKIPTNEETCDDRKEYMNQWSCGSARTMKRGYKNDNYELCKYNGVDVKPTTVRSNSSKLDAASAGTGALASSAPSTAVAQSATPSVSSSISSLRAATSGATAAASAAAAVDTGSGGGGQPHDTAPRGARKKQ

SEQ ID NO: 84 - protein, 5 aa, artificial
  glycine-serine linker
  VARIANT (1)..(5): Can be repeated between 2 and 10, inclusive
GGGGS

SEQ ID NO: 85 - protein, 5 aa, artificial
  Glycine-serine linker
  VARIANT (1)..(5): Can be repeated between 2 and 6, inclusive
GGGGS

SEQ ID NO: 86 - protein, 30 aa, artificial
  glycine-serine linker
GGGGSGGGGSGGGGSGGGGSGGGGSGGGGS